European Patent Application EP 4 194 002 A1, published June 14, 2023. Title: TGF-β RII MUTANT AND FUSION PROTEIN THEREOF. Applicant: MABWELL (SHANGHAI) BIOSCIENCE CO., LTD. The sequence listing filed with the application follows.

SEQUENCE LISTING (49 sequences)

SEQ ID NO: 1 - DNA, 1344 bp, Artificial Sequence
gaggtgcagctggtgcagtccggagccgaggtgaagaagcctggagccaccgtgaagatctcctgcaaggtgtccggcttcaacatcaaggacatctacatgcactgggtgcagcaggctcctggcaagggcctggagtggatgggacggatcgaccctgccaacgccaacaccaagtacgaccccaagttccaggaccgggtgaccatcaccgctgacacctccaccaacaccgcctacatggagctgtcctccctgcggtccgaggacaccgctgtgtactactgcgcctctggccagctgggacctctgggcttcgactactggggacagggcaccaccgtgaccgtgtcctccgctagcaccaagggcccatcggtcttccccctggcaccctcctccaagagcacctctgggggcacagcggccctgggctgcctggtcaaggactacttccccgaaccggtgacggtgtcgtggaactcaggcgccctgaccagcggcgtgcacaccttcccggctgtcctacagtcctcaggactctactccctcagcagcgtggtgaccgtgccctccagcagcttgggcacccagacctacatctgcaacgtgaatcacaagcccagcaacaccaaggtggacaagaaagttgagcccaaatcttgtgacaaaactcacacatgcccaccgtgcccagcacctgaactcctggggggaccgtcagtcttcctcttccccccaaaacccaaggacaccctcatgatctcccggacccctgaggtcacatgcgtggtggtggacgtgagccacgaagaccctgaggtcaagttcaactggtacgtggacggcgtggaggtgcataatgccaagacaaagccgcgggaggagcagtacaacagcacgtaccgtgtggtcagcgtcctcaccgtcctgcaccaggactggctgaatggcaaggagtacaagtgcaaggtctccaacaaagccctcccagcccccatcgagaaaaccatctccaaagccaaagggcagccccgagaaccacaggtgtacaccctgcctccatctcgggatgagctgaccaagaaccaggtcagcctgacctgcctggtcaaaggcttctatcccagcgacatcgccgtggagtgggagagcaatgggcagccggagaacaactacaagaccacgcctcccgtgctggactccgacggctccttcttcctctatagcaagctcaccgtggacaagagcaggtggcagcaggggaacgtcttctcatgctccgtgatgcatgaggctctgcacaaccactacacgcagaagagcctctccctgtctccgggt

SEQ ID NO: 2 - protein, 448 aa, Artificial Sequence
EVQLVQSGAEVKKPGATVKISCKVSGFNIKDIYMHWVQQAPGKGLEWMGRIDPANANTKYDPKFQDRVTITADTSTNTAYMELSSLRSEDTAVYYCASGQLGPLGFDYWGQGTTVTVSSASTKGPSVFPLAPSSKSTSGGTAALGCLVKDYFPEPVTVSWNSGALTSGVHTFPAVLQSSGLYSLSSVVTVPSSSLGTQTYICNVNHKPSNTKVDKKVEPKSCDKTHTCPPCPAPELLGGPSVFLFPPKPKDTLMISRTPEVTCVVVDVSHEDPEVKFNWYVDGVEVHNAKTKPREEQYNSTYRVVSVLTVLHQDWLNGKEYKCKVSNKALPAPIEKTISKAKGQPREPQVYTLPPSRDELTKNQVSLTCLVKGFYPSDIAVEWESNGQPENNYKTTPPVLDSDGSFFLYSKLTVDKSRWQQGNVFSCSVMHEALHNHYTQKSLSLSPG

SEQ ID NO: 3 - DNA, 66 bp, Artificial Sequence
gctggtggaggtggctccggaggcggaggatctggaggaggtggcagcggcggtggaggctctggt

SEQ ID NO: 4 - protein, 22 aa, Artificial Sequence
AGGGGSGGGGSGGGGSGGGGSG

SEQ ID NO: 5 - DNA, 408 bp, Artificial Sequence
atccctccacacgtgcagaagtccgtgaacaacgacatgatcgtgaccgacaacaacggagccgtgaagttccctcagctgtgcaagttctgcgacgtgcggttctccacctgcgacaaccagaagtcctgcatgtccaactgctccatcacctccatctgcgagaagcctcaggaggtgtgcgtggccgtgtggcggaagaacgacgagaacatcaccctggagaccgtgtgccacgaccctaagctgccctaccacgacttcatcctggaggacgctgcctctcccaagtgcatcatgaaggagaagaagaagcctggcgagaccttcttcatgtgctcctgctcctccgacgagtgcaacgacaacatcatcttctccgaggagtacaacacctccaaccctgac

SEQ ID NO: 6 - protein, 136 aa, Artificial Sequence
IPPHVQKSVNNDMIVTDNNGAVKFPQLCKFCDVRFSTCDNQKSCMSNCSITSICEKPQEVCVAVWRKNDENITLETVCHDPKLPYHDFILEDAASPKCIMKEKKKPGETFFMCSCSSDECNDNIIFSEEYNTSNPD

SEQ ID NO: 7 - DNA, 642 bp, Artificial Sequence
gacatccagatgacccagtctccctcctctctgtctgcctccgtgggcgacagagtgaccatcacctgcagagcctcccaggacatctccaactacctgaactggtaccagcagaagcctggcaaggctcccaagctgctgctgtactacacctccaggctgcactccggagtgccctctcggttctctggctccggctctggcaccgactacaccctgaccatctcctccctgcagcccgaggacttcgccacctacttctgccagcagggcgctggacggccctacaccttcggaggaggcaccaaggtggagatcaagcggaccgtggcggcgccatctgtcttcatcttcccgccatctgatgagcagttgaaatctggtaccgctagcgttgtgtgcctgctgaataacttctatcccagagaggccaaagtacagtggaaggtggataacgccctccaatcgggtaactcccaggagagtgtcacagagcaggacagcaaggacagcacctacagcctcagcagcaccctgacgctgagcaaagcagactacgagaaacacaaagtctacgcctgcgaagtcacccatcagggcctgagctcgcccgtcacaaagagcttcaacaggggagagtgt

SEQ ID NO: 8 - protein, 214 aa, Artificial Sequence
DIQMTQSPSSLSASVGDRVTITCRASQDISNYLNWYQQKPGKAPKLLLYYTSRLHSGVPSRFSGSGSGTDYTLTISSLQPEDFATYFCQQGAGRPYTFGGGTKVEIKRTVAAPSVFIFPPSDEQLKSGTASVVCLLNNFYPREAKVQWKVDNALQSGNSQESVTEQDSKDSTYSLSSTLTLSKADYEKHKVYACEVTHQGLSSPVTKSFNRGEC

SEQ ID NO: 9 - DNA, 1818 bp, Artificial Sequence
gaggtgcagctggtgcagtccggagccgaggtgaagaagcctggagccaccgtgaagatctcctgcaaggtgtccggcttcaacatcaaggacatctacatgcactgggtgcagcaggctcctggcaagggcctggagtggatgggacggatcgaccctgccaacgccaacaccaagtacgaccccaagttccaggaccgggtgaccatcaccgctgacacctccaccaacaccgcctacatggagctgtcctccctgcggtccgaggacaccgctgtgtactactgcgcctctggccagctgggacctctgggcttcgactactggggacagggcaccaccgtgaccgtgtcctccgctagcaccaagggcccatcggtcttccccctggcaccctcctccaagagcacctctgggggcacagcggccctgggctgcctggtcaaggactacttccccgaaccggtgacggtgtcgtggaactcaggcgccctgaccagcggcgtgcacaccttcccggctgtcctacagtcctcaggactctactccctcagcagcgtggtgaccgtgccctccagcagcttgggcacccagacctacatctgcaacgtgaatcacaagcccagcaacaccaaggtggacaagaaagttgagcccaaatcttgtgacaaaactcacacatgcccaccgtgcccagcacctgaactcctggggggaccgtcagtcttcctcttccccccaaaacccaaggacaccctcatgatctcccggacccctgaggtcacatgcgtggtggtggacgtgagccacgaagaccctgaggtcaagttcaactggtacgtggacggcgtggaggtgcataatgccaagacaaagccgcgggaggagcagtacaacagcacgtaccgtgtggtcagcgtcctcaccgtcctgcaccaggactggctgaatggcaaggagtacaagtgcaaggtctccaacaaagccctcccagcccccatcgagaaaaccatctccaaagccaaagggcagccccgagaaccacaggtgtacaccctgcctccatctcgggatgagctgaccaagaaccaggtcagcctgacctgcctggtcaaaggcttctatcccagcgacatcgccgtggagtgggagagcaatgggcagccggagaacaactacaagaccacgcctcccgtgctggactccgacggctccttcttcctctatagcaagctcaccgtggacaagagcaggtggcagcaggggaacgtcttctcatgctccgtgatgcatgaggctctgcacaaccactacacgcagaagagcctctccctgtctccgggtgctggtggaggtggctccggaggcggaggatctggaggaggtggcagcggcggtggaggctctggtatccctccacacgtgcagaagtccgtgaacaacgacatgatcgtgaccgacaacaacggagccgtgaagttccctcagctgtgcaagttctgcgacgtgcggttctccacctgcgacaaccagaagtcctgcatgtccaactgctccatcacctccatctgcgagaagcctcaggaggtgtgcgtggccgtgtggcggaagaacgacgagaacatcaccctggagaccgtgtgccacgaccctaagctgccctaccacgacttcatcctggaggacgctgcctctcccaagtgcatcatgaaggagaagaagaagcctggcgagaccttcttcatgtgctcctgctcctccgacgagtgcaacgacaacatcatcttctccgaggagtacaacacctccaaccctgac

SEQ ID NO: 10 - protein, 606 aa, Artificial Sequence
EVQLVQSGAEVKKPGATVKISCKVSGFNIKDIYMHWVQQAPGKGLEWMGRIDPANANTKYDPKFQDRVTITADTSTNTAYMELSSLRSEDTAVYYCASGQLGPLGFDYWGQGTTVTVSSASTKGPSVFPLAPSSKSTSGGTAALGCLVKDYFPEPVTVSWNSGALTSGVHTFPAVLQSSGLYSLSSVVTVPSSSLGTQTYICNVNHKPSNTKVDKKVEPKSCDKTHTCPPCPAPELLGGPSVFLFPPKPKDTLMISRTPEVTCVVVDVSHEDPEVKFNWYVDGVEVHNAKTKPREEQYNSTYRVVSVLTVLHQDWLNGKEYKCKVSNKALPAPIEKTISKAKGQPREPQVYTLPPSRDELTKNQVSLTCLVKGFYPSDIAVEWESNGQPENNYKTTPPVLDSDGSFFLYSKLTVDKSRWQQGNVFSCSVMHEALHNHYTQKSLSLSPGAGGGGSGGGGSGGGGSGGGGSGIPPHVQKSVNNDMIVTDNNGAVKFPQLCKFCDVRFSTCDNQKSCMSNCSITSICEKPQEVCVAVWRKNDENITLETVCHDPKLPYHDFILEDAASPKCIMKEKKKPGETFFMCSCSSDECNDNIIFSEEYNTSNPD

SEQ ID NO: 11 - DNA, 1818 bp, Artificial Sequence
gaggtgcagctggtgcagtccggagccgaggtgaagaagcctggagccaccgtgaagatctcctgcaaggtgtccggcttcaacatcaaggacatctacatgcactgggtgcagcaggctcctggcaagggcctggagtggatgggacggatcgaccctgccaacgccaacaccaagtacgaccccaagttccaggaccgggtgaccatcaccgctgacacctccaccaacaccgcctacatggagctgtcctccctgcggtccgaggacaccgctgtgtactactgcgcctctggccagctgggacctctgggcttcgactactggggacagggcaccaccgtgaccgtgtcctccgctagcaccaagggcccatcggtcttccccctggcaccctcctccaagagcacctctgggggcacagcggccctgggctgcctggtcaaggactacttccccgaaccggtgacggtgtcgtggaactcaggcgccctgaccagcggcgtgcacaccttcccggctgtcctacagtcctcaggactctactccctcagcagcgtggtgaccgtgccctccagcagcttgggcacccagacctacatctgcaacgtgaatcacaagcccagcaacaccaaggtggacaagaaagttgagcccaaatcttgtgacaaaactcacacatgcccaccgtgcccagcacctgaactcctggggggaccgtcagtcttcctcttccccccaaaacccaaggacaccctcatgatctcccggacccctgaggtcacatgcgtggtggtggacgtgagccacgaagaccctgaggtcaagttcaactggtacgtggacggcgtggaggtgcataatgccaagacaaagccgcgggaggagcagtacaacagcacgtaccgtgtggtcagcgtcctcaccgtcctgcaccaggactggctgaatggcaaggagtacaagtgcaaggtctccaacaaagccctcccagcccccatcgagaaaaccatctccaaagccaaagggcagccccgagaaccacaggtgtacaccctgcctccatctcgggatgagctgaccaagaaccaggtcagcctgacctgcctggtcaaaggcttctatcccagcgacatcgccgtggagtgggagagcaatgggcagccggagaacaactacaagaccacgcctcccgtgctggactccgacggctccttcttcctctatagcaagctcaccgtggacaagagcaggtggcagcaggggaacgtcttctcatgctccgtgatgcatgaggctctgcacaaccactacacgcagaagagcctctccctgtctccgggtgctggtggaggtggctccggaggcggaggatctggaggaggtggcagcggcggtggaggctctggtatccctccacacgtgcagaagtccgtgaacaacgacatgatcgtgaccgacaacaacaccgccgtgaagttccctcagctgtgcaagttctgcgacgtgcggttctccacctgcgacaaccagaagtcctgcatgtccaactgctccatcacctccatctgcgagaagcctcaggaggtgtgcgtggccgtgtggcggaagaacgacgagaacatcaccctggagaccgtgtgccacgaccctaagctgccctaccacgacttcatcctggaggacgctgcctctcccaagtgcatcatgaaggagaagaagaagcctggcgagaccttcttcatgtgctcctgctcctccgacgagtgcaacgacaacatcatcttctccgaggagtacaacacctccaaccctgac

SEQ ID NO: 12 - protein, 606 aa, Artificial Sequence
EVQLVQSGAEVKKPGATVKISCKVSGFNIKDIYMHWVQQAPGKGLEWMGRIDPANANTKYDPKFQDRVTITADTSTNTAYMELSSLRSEDTAVYYCASGQLGPLGFDYWGQGTTVTVSSASTKGPSVFPLAPSSKSTSGGTAALGCLVKDYFPEPVTVSWNSGALTSGVHTFPAVLQSSGLYSLSSVVTVPSSSLGTQTYICNVNHKPSNTKVDKKVEPKSCDKTHTCPPCPAPELLGGPSVFLFPPKPKDTLMISRTPEVTCVVVDVSHEDPEVKFNWYVDGVEVHNAKTKPREEQYNSTYRVVSVLTVLHQDWLNGKEYKCKVSNKALPAPIEKTISKAKGQPREPQVYTLPPSRDELTKNQVSLTCLVKGFYPSDIAVEWESNGQPENNYKTTPPVLDSDGSFFLYSKLTVDKSRWQQGNVFSCSVMHEALHNHYTQKSLSLSPGAGGGGSGGGGSGGGGSGGGGSGIPPHVQKSVNNDMIVTDNNTAVKFPQLCKFCDVRFSTCDNQKSCMSNCSITSICEKPQEVCVAVWRKNDENITLETVCHDPKLPYHDFILEDAASPKCIMKEKKKPGETFFMCSCSSDECNDNIIFSEEYNTSNPD

SEQ ID NO: 13 - DNA, 1818 bp, Artificial Sequence
gaggtgcagctggtgcagtccggagccgaggtgaagaagcctggagccaccgtgaagatctcctgcaaggtgtccggcttcaacatcaaggacatctacatgcactgggtgcagcaggctcctggcaagggcctggagtggatgggacggatcgaccctgccaacgccaacaccaagtacgaccccaagttccaggaccgggtgaccatcaccgctgacacctccaccaacaccgcctacatggagctgtcctccctgcggtccgaggacaccgctgtgtactactgcgcctctggccagctgggacctctgggcttcgactactggggacagggcaccaccgtgaccgtgtcctccgctagcaccaagggcccatcggtcttccccctggcaccctcctccaagagcacctctgggggcacagcggccctgggctgcctggtcaaggactacttccccgaaccggtgacggtgtcgtggaactcaggcgccctgaccagcggcgtgcacaccttcccggctgtcctacagtcctcaggactctactccctcagcagcgtggtgaccgtgccctccagcagcttgggcacccagacctacatctgcaacgtgaatcacaagcccagcaacaccaaggtggacaagaaagttgagcccaaatcttgtgacaaaactcacacatgcccaccgtgcccagcacctgaactcctggggggaccgtcagtcttcctcttccccccaaaacccaaggacaccctcatgatctcccggacccctgaggtcacatgcgtggtggtggacgtgagccacgaagaccctgaggtcaagttcaactggtacgtggacggcgtggaggtgcataatgccaagacaaagccgcgggaggagcagtacaacagcacgtaccgtgtggtcagcgtcctcaccgtcctgcaccaggactggctgaatggcaaggagtacaagtgcaaggtctccaacaaagccctcccagcccccatcgagaaaaccatctccaaagccaaagggcagccccgagaaccacaggtgtacaccctgcctccatctcgggatgagctgaccaagaaccaggtcagcctgacctgcctggtcaaaggcttctatcccagcgacatcgccgtggagtgggagagcaatgggcagccggagaacaactacaagaccacgcctcccgtgctggactccgacggctccttcttcctctatagcaagctcaccgtggacaagagcaggtggcagcaggggaacgtcttctcatgctccgtgatgcatgaggctctgcacaaccactacacgcagaagagcctctccctgtctccgggtgctggtggaggtggctccggaggcggaggatctggaggaggtggcagcggcggtggaggctctggtatccctccacacgtgaacaagtccgtgaacaacgacatgatcgtgaccgacaacaacggagccgtgaagttccctcagctgtgcaagttctgcgacgtgcggttctccacctgcgacaaccagaagtcctgcatgtccaactgctccatcacctccatctgcgagaagcctcaggaggtgtgcgtggccgtgtggcggaagaacgacgagaacatcaccctggagaccgtgtgccacgaccctaagctgccctaccacgacttcatcctggaggacgctgcctctcccaagtgcatcatgaaggagaagaagaagcctggcgagaccttcttcatgtgctcctgctcctccgacgagtgcaacgacaacatcatcttctccgaggagtacaacacctccaaccctgac

SEQ ID NO: 14 - protein, 606 aa, Artificial Sequence
EVQLVQSGAEVKKPGATVKISCKVSGFNIKDIYMHWVQQAPGKGLEWMGRIDPANANTKYDPKFQDRVTITADTSTNTAYMELSSLRSEDTAVYYCASGQLGPLGFDYWGQGTTVTVSSASTKGPSVFPLAPSSKSTSGGTAALGCLVKDYFPEPVTVSWNSGALTSGVHTFPAVLQSSGLYSLSSVVTVPSSSLGTQTYICNVNHKPSNTKVDKKVEPKSCDKTHTCPPCPAPELLGGPSVFLFPPKPKDTLMISRTPEVTCVVVDVSHEDPEVKFNWYVDGVEVHNAKTKPREEQYNSTYRVVSVLTVLHQDWLNGKEYKCKVSNKALPAPIEKTISKAKGQPREPQVYTLPPSRDELTKNQVSLTCLVKGFYPSDIAVEWESNGQPENNYKTTPPVLDSDGSFFLYSKLTVDKSRWQQGNVFSCSVMHEALHNHYTQKSLSLSPGAGGGGSGGGGSGGGGSGGGGSGIPPHVNKSVNNDMIVTDNNGAVKFPQLCKFCDVRFSTCDNQKSCMSNCSITSICEKPQEVCVAVWRKNDENITLETVCHDPKLPYHDFILEDAASPKCIMKEKKKPGETFFMCSCSSDECNDNIIFSEEYNTSNPD

SEQ ID NO: 15 - DNA, 1818 bp, Artificial Sequence
gaggtgcagctggtgcagtccggagccgaggtgaagaagcctggagccaccgtgaagatctcctgcaaggtgtccggcttcaacatcaaggacatctacatgcactgggtgcagcaggctcctggcaagggcctggagtggatgggacggatcgaccctgccaacgccaacaccaagtacgaccccaagttccaggaccgggtgaccatcaccgctgacacctccaccaacaccgcctacatggagctgtcctccctgcggtccgaggacaccgctgtgtactactgcgcctctggccagctgggacctctgggcttcgactactggggacagggcaccaccgtgaccgtgtcctccgctagcaccaagggcccatcggtcttccccctggcaccctcctccaagagcacctctgggggcacagcggccctgggctgcctggtcaaggactacttccccgaaccggtgacggtgtcgtggaactcaggcgccctgaccagcggcgtgcacaccttcccggctgtcctacagtcctcaggactctactccctcagcagcgtggtgaccgtgccctccagcagcttgggcacccagacctacatctgcaacgtgaatcacaagcccagcaacaccaaggtggacaagaaagttgagcccaaatcttgtgacaaaactcacacatgcccaccgtgcccagcacctgaactcctggggggaccgtcagtcttcctcttccccccaaaacccaaggacaccctcatgatctcccggacccctgaggtcacatgcgtggtggtggacgtgagccacgaagaccctgaggtcaagttcaactggtacgtggacggcgtggaggtgcataatgccaagacaaagccgcgggaggagcagtacaacagcacgtaccgtgtggtcagcgtcctcaccgtcctgcaccaggactggctgaatggcaaggagtacaagtgcaaggtctccaacaaagccctcccagcccccatcgagaaaaccatctccaaagccaaagggcagccccgagaaccacaggtgtacaccctgcctccatctcgggatgagctgaccaagaaccaggtcagcctgacctgcctggtcaaaggcttctatcccagcgacatcgccgtggagtgggagagcaatgggcagccggagaacaactacaagaccacgcctcccgtgctggactccgacggctccttcttcctctatagcaagctcaccgtggacaagagcaggtggcagcaggggaacgtcttctcatgctccgtgatgcatgaggctctgcacaaccactacacgcagaagagcctctccctgtctccgggtgctggtggaggtggctccggaggcggaggatctggaggaggtggcagcggcggtggaggctctggtatccctccacacgtgcagaagtccgtgaacaacaccatgatcgtgaccgacaacaacggagccgtgaagttccctcagctgtgcaagttctgcgacgtgcggttctccacctgcgacaaccagaagtcctgcatgtccaactgctccatcacctccatctgcgagaagcctcaggaggtgtgcgtggccgtgtggcggaagaacgacgagaacatcaccctggagaccgtgtgccacgaccctaagctgccctaccacgacttcatcctggaggacgctgcctctcccaagtgcatcatgaaggagaagaagaagcctggcgagaccttcttcatgtgctcctgctcctccgacgagtgcaacgacaacatcatcttctccgaggagtacaacacctccaaccctgac

SEQ ID NO: 16 - protein, 606 aa, Artificial Sequence
EVQLVQSGAEVKKPGATVKISCKVSGFNIKDIYMHWVQQAPGKGLEWMGRIDPANANTKYDPKFQDRVTITADTSTNTAYMELSSLRSEDTAVYYCASGQLGPLGFDYWGQGTTVTVSSASTKGPSVFPLAPSSKSTSGGTAALGCLVKDYFPEPVTVSWNSGALTSGVHTFPAVLQSSGLYSLSSVVTVPSSSLGTQTYICNVNHKPSNTKVDKKVEPKSCDKTHTCPPCPAPELLGGPSVFLFPPKPKDTLMISRTPEVTCVVVDVSHEDPEVKFNWYVDGVEVHNAKTKPREEQYNSTYRVVSVLTVLHQDWLNGKEYKCKVSNKALPAPIEKTISKAKGQPREPQVYTLPPSRDELTKNQVSLTCLVKGFYPSDIAVEWESNGQPENNYKTTPPVLDSDGSFFLYSKLTVDKSRWQQGNVFSCSVMHEALHNHYTQKSLSLSPGAGGGGSGGGGSGGGGSGGGGSGIPPHVQKSVNNTMIVTDNNGAVKFPQLCKFCDVRFSTCDNQKSCMSNCSITSICEKPQEVCVAVWRKNDENITLETVCHDPKLPYHDFILEDAASPKCIMKEKKKPGETFFMCSCSSDECNDNIIFSEEYNTSNPD

SEQ ID NO: 17 - protein, 216 aa, Artificial Sequence
QSALTQPASVSGSPGQSITISCTGTSSDVGGYNYVSWYQQHPGKAPKLMIYDVSNRPSGVSNRFSGSKSGNTASLTISGLQAEDEADYYCSSYTSSSTRVFGTGTKVTVLGQPKANPTVTLFPPSSEELQANKATLVCLISDFYPGAVTVAWKADGSPVKAGVETTKPSKQSNNKYAASSYLSLTPEQWKSHRSYSCQVTHEGSTVEKTVAPTECS

SEQ ID NO: 18 - protein, 607 aa, Artificial Sequence
EVQLLESGGGLVQPGGSLRLSCAASGFTFSSYIMMWVRQAPGKGLEWVSSIYPSGGITFYADTVKGRFTISRDNSKNTLYLQMNSLRAEDTAVYYCARIKLGTVTTVDYWGQGTLVTVSSASTKGPSVFPLAPSSKSTSGGTAALGCLVKDYFPEPVTVSWNSGALTSGVHTFPAVLQSSGLYSLSSVVTVPSSSLGTQTYICNVNHKPSNTKVDKKVEPKSCDKTHTCPPCPAPELLGGPSVFLFPPKPKDTLMISRTPEVTCVVVDVSHEDPEVKFNWYVDGVEVHNAKTKPREEQYNSTYRVVSVLTVLHQDWLNGKEYKCKVSNKALPAPIEKTISKAKGQPREPQVYTLPPSRDELTKNQVSLTCLVKGFYPSDIAVEWESNGQPENNYKTTPPVLDSDGSFFLYSKLTVDKSRWQQGNVFSCSVMHEALHNHYTQKSLSLSPGAGGGGSGGGGSGGGGSGGGGSGIPPHVQKSVNNDMIVTDNNGAVKFPQLCKFCDVRFSTCDNQKSCMSNCSITSICEKPQEVCVAVWRKNDENITLETVCHDPKLPYHDFILEDAASPKCIMKEKKKPGETFFMCSCSSDECNDNIIFSEEYNTSNPD

SEQ ID NO: 19 - DNA, 1059 bp, Artificial Sequence
gaggtgcagctggtggagtctggaggtggcctggtgcagcctggaggctccctgaggctgtcctgcgctgcctctcgggactccgacgagggagcctcctgcatgggctggttcaggcaggctcctggcaaggagagagagggagtggccatcatcttcaacgctggcgagcggaccgactacggcgactccgtgaagggacggttcaccatctccagggacaacgccaagaacaccctgtacctgcagatgaactccctgagagccgaggacacagccgtgtactactgcgctaccgtgtggtgtggctcctgggtggctcggtcctggggacagggcaccctggtgaccgtgtcctccgctagcgagcccaaatctagcgacaaaactcacacatgcccaccgtgcccagcacctgaactcctggggggaccgtcagtcttcctcttccccccaaaacccaaggacaccctcatgatctcccggacccctgaggtcacatgcgtggtggtggacgtgagccacgaagaccctgaggtcaagttcaactggtacgtggacggcgtggaggtgcataatgccaagacaaagccgcgggaggagcagtacaacagcacgtaccgtgtggtcagcgtcctcaccgtcctgcaccaggactggctgaatggcaaggagtacaagtgcaaggtctccaacaaagccctcccagcccccatcgagaaaaccatctccaaagccaaagggcagccccgagaaccacaggtgtacaccctgcctccatctcgggatgagctgaccaagaaccaggtcagcctgacctgcctggtcaaaggcttctatcccagcgacatcgccgtggagtgggagagcaatgggcagccggagaacaactacaagaccacgcctcccgtgctggactccgacggctccttcttcctctatagcaagctcaccgtggacaagagcaggtggcagcaggggaacgtcttctcatgctccgtgatgcatgaggctctgcacaaccactacacgcagaagagcctctccctgtccccgggt

SEQ ID NO: 20 - protein, 353 aa, Artificial Sequence
EVQLVESGGGLVQPGGSLRLSCAASRDSDEGASCMGWFRQAPGKEREGVAIIFNAGERTDYGDSVKGRFTISRDNAKNTLYLQMNSLRAEDTAVYYCATVWCGSWVARSWGQGTLVTVSSASEPKSSDKTHTCPPCPAPELLGGPSVFLFPPKPKDTLMISRTPEVTCVVVDVSHEDPEVKFNWYVDGVEVHNAKTKPREEQYNSTYRVVSVLTVLHQDWLNGKEYKCKVSNKALPAPIEKTISKAKGQPREPQVYTLPPSRDELTKNQVSLTCLVKGFYPSDIAVEWESNGQPENNYKTTPPVLDSDGSFFLYSKLTVDKSRWQQGNVFSCSVMHEALHNHYTQKSLSLSPG

SEQ ID NO: 21 - DNA, 63 bp, Artificial Sequence
ggtggaggtggctccggaggcggaggatctggaggaggtggcagcggcggtggaggctctggt

SEQ ID NO: 22 - protein, 21 aa, Artificial Sequence
GGGGSGGGGSGGGGSGGGGSG

SEQ ID NO: 23 - DNA, 1530 bp, Artificial Sequence
gaggtgcagctggtggagtctggaggtggcctggtgcagcctggaggctccctgaggctgtcctgcgctgcctctcgggactccgacgagggagcctcctgcatgggctggttcaggcaggctcctggcaaggagagagagggagtggccatcatcttcaacgctggcgagcggaccgactacggcgactccgtgaagggacggttcaccatctccagggacaacgccaagaacaccctgtacctgcagatgaactccctgagagccgaggacacagccgtgtactactgcgctaccgtgtggtgtggctcctgggtggctcggtcctggggacagggcaccctggtgaccgtgtcctccgctagcgagcccaaatctagcgacaaaactcacacatgcccaccgtgcccagcacctgaactcctggggggaccgtcagtcttcctcttccccccaaaacccaaggacaccctcatgatctcccggacccctgaggtcacatgcgtggtggtggacgtgagccacgaagaccctgaggtcaagttcaactggtacgtggacggcgtggaggtgcataatgccaagacaaagccgcgggaggagcagtacaacagcacgtaccgtgtggtcagcgtcctcaccgtcctgcaccaggactggctgaatggcaaggagtacaagtgcaaggtctccaacaaagccctcccagcccccatcgagaaaaccatctccaaagccaaagggcagccccgagaaccacaggtgtacaccctgcctccatctcgggatgagctgaccaagaaccaggtcagcctgacctgcctggtcaaaggcttctatcccagcgacatcgccgtggagtgggagagcaatgggcagccggagaacaactacaagaccacgcctcccgtgctggactccgacggctccttcttcctctatagcaagctcaccgtggacaagagcaggtggcagcaggggaacgtcttctcatgctccgtgatgcatgaggctctgcacaaccactacacgcagaagagcctctccctgtccccgggtggtggaggtggctccggaggcggaggatctggaggaggtggcagcggcggtggaggctctggtatccctccacacgtgaacaagtccgtgaacaacgacatgatcgtgaccgacaacaacggagccgtgaagttccctcagctgtgcaagttctgcgacgtgcggttctccacctgcgacaaccagaagtcctgcatgtccaactgctccatcacctccatctgcgagaagcctcaggaggtgtgcgtggccgtgtggcggaagaacgacgagaacatcaccctggagaccgtgtgccacgaccctaagctgccctaccacgacttcatcctggaggacgctgcctctcccaagtgcatcatgaaggagaagaagaagcctggcgagaccttcttcatgtgctcctgctcctccgacgagtgcaacgacaacatcatcttctccgaggagtacaacacctccaaccctgac

SEQ ID NO: 24 - protein, 510 aa, Artificial Sequence
EVQLVESGGGLVQPGGSLRLSCAASRDSDEGASCMGWFRQAPGKEREGVAIIFNAGERTDYGDSVKGRFTISRDNAKNTLYLQMNSLRAEDTAVYYCATVWCGSWVARSWGQGTLVTVSSASEPKSSDKTHTCPPCPAPELLGGPSVFLFPPKPKDTLMISRTPEVTCVVVDVSHEDPEVKFNWYVDGVEVHNAKTKPREEQYNSTYRVVSVLTVLHQDWLNGKEYKCKVSNKALPAPIEKTISKAKGQPREPQVYTLPPSRDELTKNQVSLTCLVKGFYPSDIAVEWESNGQPENNYKTTPPVLDSDGSFFLYSKLTVDKSRWQQGNVFSCSVMHEALHNHYTQKSLSLSPGGGGGSGGGGSGGGGSGGGGSGIPPHVNKSVNNDMIVTDNNGAVKFPQLCKFCDVRFSTCDNQKSCMSNCSITSICEKPQEVCVAVWRKNDENITLETVCHDPKLPYHDFILEDAASPKCIMKEKKKPGETFFMCSCSSDECNDNIIFSEEYNTSNPD

SEQ ID NO: 25 - protein, 5 aa, Artificial Sequence
DIYMH

SEQ ID NO: 26 - protein, 17 aa, Artificial Sequence
RIDPANANTKYDPKFQD

SEQ ID NO: 27 - protein, 10 aa, Artificial Sequence
GQLGPLGFDY

SEQ ID NO: 28 - protein, 11 aa, Artificial Sequence
RASQDISNYLN

SEQ ID NO: 29 - protein, 7 aa, Artificial Sequence
YTSRLHS

SEQ ID NO: 30 - protein, 9 aa, Artificial Sequence
QQGAGRPYT

SEQ ID NO: 31 - protein, 16 aa, Artificial Sequence
VVSVLTVLHQDWLNGK

SEQ ID NO: 32 - protein, 23 aa, Artificial Sequence
WQQGNVFSCSVMHEALHNHYTQK

SEQ ID NO: 33 - protein, 10 aa, Artificial Sequence
NQVSLTCLVK

SEQ ID NO: 34 - protein, 14 aa, Artificial Sequence
FNWYVDGVEVHNAK

SEQ ID NO: 35 - protein, 7 aa, Artificial Sequence
DTLMISR

SEQ ID NO: 36 - protein, 12 aa, Artificial Sequence
GPSVFPLAPSSK

SEQ ID NO: 37 - protein, 12 aa, Artificial Sequence
EVQLVQSGAEVK

SEQ ID NO: 38 - protein, 20 aa, Artificial Sequence
VTITADTSTNTAYMELSSLR

SEQ ID NO: 39 - protein, 13 aa, Artificial Sequence
DIYMHWVQQAPGK

SEQ ID NO: 40 - protein, 11 aa, Artificial Sequence
EPQVYTLPPSR

SEQ ID NO: 41 - protein, 7 aa, Artificial Sequence
GLEWMGR

SEQ ID NO: 42 - protein, 8 aa, Artificial Sequence
ALPAPIEK

SEQ ID NO: 43 - protein, 26 aa, Artificial Sequence
THTCPPCPAPELLGGPSVFLFPPKPK

SEQ ID NO: 44 - protein, 22 aa, Artificial Sequence
GFYPSDIAVEWESNGQPENNYK

SEQ ID NO: 45 - protein, 16 aa, Artificial Sequence
EPQVYTLPPSRDELTK

SEQ ID NO: 46 - protein, 17 aa, Artificial Sequence
TTPPVLDSDGSFFLYSK

SEQ ID NO: 47 - protein, 9 aa, Artificial Sequence
IDPANANTK

SEQ ID NO: 48 - protein, 36 aa, Artificial Sequence
SLSLSPGAGGGGSGGGGSGGGGSGGGGSGIPPHVQK

SEQ ID NO: 49 - protein, 30 aa, Artificial Sequence
SCDKTHTCPPCPAPELLGGPSVFLFPPKPK